European Patent Specification EP 3 811 967 B1, published December 20, 2023. Title: Preparation of Biologically Active Complexes. Applicant: Hamlet Pharma AB. The sequence listing filed with the application follows.

SEQUENCE LISTING (7 sequences)

SEQ ID NO: 1 - protein, 40 aa, Artificial Sequence
  Mutated protein fragment
  SITE (6)..(6): any amino acid other than Cys
  SITE (28)..(28): any amino acid other than Cys
KQFTKXELSQLLKDIDGYGGIALPELIXTMFHTSGYDTQA

SEQ ID NO: 2 - protein, 43 aa, Artificial Sequence
  Mutated protein fragment
  SITE (11)..(11): any amino acid other than Cys
  SITE (31)..(31): any amino acid other than Cys
  SITE (40)..(40): any amino acid other than Cys
LDDDITDDIMXAKKILDIKGIDYWLAHKALXTEKLEQWLXEKL

SEQ ID NO: 3 - protein, 40 aa, Artificial Sequence
  Mutated protein fragment
KQFTKAELSQLLKDIDGYGGIALPELIATMFHTSGYDTQA

SEQ ID NO: 4 - protein, 43 aa, Artificial Sequence
  Mutated protein fragment
LDDDITDDIMAAKKILDIKGIDYWLAHKALATEKLEQWLAEKL

SEQ ID NO: 5 - protein, 23 aa, Artificial Sequence
  Protein fragment
MAGWDIFGWFRDVLASLGLWNKH

SEQ ID NO: 6 - protein, 39 aa, Artificial Sequence
  Mutated protein fragment
  SITE (6)..(6): any amino acid other than Cys
  SITE (28)..(28): any amino acid other than Cys
KQFTKXELSQLLKDIDGYGGIALPELIXTMFHTSGYDTQ

SEQ ID NO: 7 - protein, 39 aa, Artificial Sequence
  Mutated protein fragment
KQFTKAELSQLLKDIDGYGGIALPELIATMFHTSGYDTQ